European Patent Application EP 4 656 717 A1, published December 3, 2025. Title: Glucose Oxidase Mutant, Method for Preparing, and Uses. Applicant: Shanghai United Imaging Microelectronics Technology Co., Ltd. Application EP. The sequence listing filed with the application follows.

SEQUENCE LISTING (17 sequences)

SEQ ID NO: 1 - protein, 605 aa, synthetic construct
MQTLLVSSLVVSLAAALPHYIRSNGIEASLLTDPKDVSGRTVDYIIAGGGLTGLTTAARLTENPNISVLVIESGSYESDRGPIIEDLNAYGDIFGSSVDHAYETVELATNNQTALIRSGNGLGGSTLVNGGTWTRPHKAQVDSWETVFGNEGWNWDNVAAYSLQAERARAPNAKQIAAGHYFNASCHGVNGTVHAGPRDTGDDYSPIVKALMSAVEDRGVPTKKDFGCGDPHGVSMFPNTLHEDQVRSDAAREWLLPNYQRPNLQVLTGQYVGKVLLSQNGTTPRAVGVEFGTHKGNTHNVYAKHEVLLAAGSAVSPTILEYSGIGMKSILEPLGIDTVVDLPVGLNLQDQTTATVRSRITSAGAGQGQAAWFATFNETFGDYSEKAHELLNTKLEQWAEEAVARGGFHNTTALLIQYENYRDWIVNHNVAYSELFLDTAGVASFDVWDLLPFTRGYVHILDKDPYLHHFAYDPQYFLNELDLLGQAAATQLARNISNSGAMQTYFAGETIPGDNLAYDADLSAWTEYIPYHFRPNYHGVGTCSMMPKEMGGVVDNAARVYGVQGLRVIDGSIPPTQMSSHVMTVFYAMALKISDAILEDYASMQ

SEQ ID NO: 2 - protein, 605 aa, synthetic construct
MQTLLVSSLVVSLAAALPHYIRSNGIEASLLTDPKDVSGRTVDYIIAGGGLTGLTTAARLTENPNISVLVIESGSYESDRGPIIEDLNAYGDIFGSSVDHAYETVELATNNQTALIRSGNGLGGSTLVNKGTWTRPHKAQVDSWETVFGNEGWNWDNVAAYSLQAERARAPNAKQIAAGHYFNASCHGVNGTVHAGPRDTGDDYSPIVKALMSAVEDRGVPTKKDFGCGDPHGVSMFPNTLHEDQVRSDAAREWLLPNYQRPNLQVLTGQYVGKVLLSQNGTTPRAVGVEFGTHKGNTHNVYAKHEVLLAAGSAVSPTILEYSGIGMKSILEPLGIDTVVDLPVGLNLQDQTTATVRSRITSAGAGQGQAAWFATFNETFGDYSEKAHELLNTKLEQWAEEAVARGGFHNTTALLIQYENYRDWIVNHNVAYSELFLDTAKVASFDVWDLLPFTRGYVHILDKDPYLHHFAYDPQYFLNELDLLGQAAATQLARNISNSGAMQTYFAGETIPGDNLAYDADLSAWTEYIPYHFRPNYHGVGTCSMMPKEMGGVVDNAARVYGVQGLRVIDGSIPPTQMSSHVMTVFYAMALKISDAILEDYASMQ

SEQ ID NO: 3 - protein, 605 aa, synthetic construct
MQTLLVSSLVVSLAAALPHYIRSNGIEASLLTDPKDVSGRTVDYIIAGGGLTGLTTAARLTENPNISVLVIESGSYESDRGPIIEDLNAYGDIFGSSVDHAYETVELATNNQTALIRSGNGLGGSTLVNDGTWTRPHKAQVDSWETVFGNEGWNWDNVAAYSLQAERARAPNAKQIAAGHYFNASCHGVNGTVHAGPRDTGDDYSPIVKALMSAVEDRGVPTKKDFGCGDPHGVSMFPNTLHEDQVRSDAAREWLLPNYQRPNLQVLTGQYVGKVLLSQNGTTPRAVGVEFGTHKGNTHNVYAKHEVLLAAGSAVSPTILEYSGIGMKSILEPLGIDTVVDLPVGLNLQDQTTATVRSRITSAGAGQGQAAWFATFNETFGDYSEKAHELLNTKLEQWAEEAVARGGFHNTTALLIQYENYRDWIVNHNVAYSELFLDTADVASFDVWDLLPFTRGYVHILDKDPYLHHFAYDPQYFLNELDLLGQAAATQLARNISNSGAMQTYFAGETIPGDNLAYDADLSAWTEYIPYHFRPNYHGVGTCSMMPKEMGGVVDNAARVYGVQGLRVIDGSIPPTQMSSHVMTVFYAMALKISDAILEDYASMQ

SEQ ID NO: 4 - DNA, 1743 bp, synthetic construct
  source 1..1743: mol_type = other DNA
atgcagactctccttgtgagctcgcttgtggtctccctcgctgcggccctgccacactacatcaggagcaatggcattgaagccagcctcctgactgatcccaaggatgtctccggccgcacggtcgactacatcatcgctggtggaggtctgactggactcaccaccgctgctcgtctgacggagaaccccaacatcagtgtgctcgtcatcgaaagtggctcctacgagtcggacagaggtcctatcattgaggacctgaacgcctacggcgacatctttggcagcagtgtagaccacgcctacgagaccgtggagctcgctaccaacaatcaaaccgcgctgatccgctccggaaatggtctcggtggctctactctagtgaataaaggcacctggactcgcccccacaaggcacaggttgactcttgggagactgtctttggaaatgagggctggaactgggacaatgtggccgcctactccctccaggctgagcgtgctcgcgcaccaaatgccaaacagatcgctgctggccactacttcaacgcatcctgccatggtgttaatggtactgtccatgccggaccccgcgacaccggcgatgactattctcccatcgtcaaggctctcatgagcgctgtcgaagaccggggcgttcccaccaagaaagacttcggatgcggtgacccccatggtgtgtccatgttccccaacaccttgcacgaagaccaatatgttggtaaggtgctccttagccagaacggcaccacccctcgtgccgttggcgtggaattcggcacccacaagggcaacacccacaacgtttacgctaagcacgaggtcctcctggccgcgggctccgctgtctctcccacaatcctcgaatattccggtatcggaatgaagtccatcctggagccccttggtatcgacaccgtcgttgacctgcccgtcggcttgaacctgcaggaccagaccaccgctaccgtccgctcccgcatcacctctgctggtgcaggacagggacaggccgcttggttcgccaccttcaacgagacctttggtgactattccgaaaaggcacacgagctgctcaacaccaagctggagcagtgggccgaagaggccgtcgcccgtggcggattccacaacaccaccgccttgctcatccagtacgagaactaccgcgactggattgtcaaccacaacgtcgcgtactcggaactcttcctcgacactgccaaagtagccagcttcgatgtgtgggaccttctgcccttcacccgaggatacgttcacatcctcgacaaggacccctaccttcaccacttcgcctacgaccctcagtacttcctcaacgagctggacctgctcggtcaggctgccgctactcaactggcccgcaacatctccaactccggtgccatgcagacctacttcgctggggagactatccccggtgataacctcgcgtatgatgccgatttgagcgcctggactgagtacatcccgtaccacttccgtcctaactaccatggcgtgggtacttgctccatgatgccgaaggagatgggcggtgttgttgataatgctgcccgtgtgtatggtgtgcagggactgcgtgtcattgatggttctattcctcctacgcaaatgtcgtcccatgtcatgacggtgttctatgccatggcgctaaaaatttcggatgctatcttggaagattatgcttccatgcagtga

SEQ ID NO: 5 - DNA, 1743 bp, synthetic construct
  source 1..1743: mol_type = other DNA
atgcagactctccttgtgagctcgcttgtggtctccctcgctgcggccctgccacactacatcaggagcaatggcattgaagccagcctcctgactgatcccaaggatgtctccggccgcacggtcgactacatcatcgctggtggaggtctgactggactcaccaccgctgctcgtctgacggagaaccccaacatcagtgtgctcgtcatcgaaagtggctcctacgagtcggacagaggtcctatcattgaggacctgaacgcctacggcgacatctttggcagcagtgtagaccacgcctacgagaccgtggagctcgctaccaacaatcaaaccgcgctgatccgctccggaaatggtctcggtggctctactctagtgaatgacggcacctggactcgcccccacaaggcacaggttgactcttgggagactgtctttggaaatgagggctggaactgggacaatgtggccgcctactccctccaggctgagcgtgctcgcgcaccaaatgccaaacagatcgctgctggccactacttcaacgcatcctgccatggtgttaatggtactgtccatgccggaccccgcgacaccggcgatgactattctcccatcgtcaaggctctcatgagcgctgtcgaagaccggggcgttcccaccaagaaagacttcggatgcggtgacccccatggtgtgtccatgttccccaacaccttgcacgaagaccaatatgttggtaaggtgctccttagccagaacggcaccacccctcgtgccgttggcgtggaattcggcacccacaagggcaacacccacaacgtttacgctaagcacgaggtcctcctggccgcgggctccgctgtctctcccacaatcctcgaatattccggtatcggaatgaagtccatcctggagccccttggtatcgacaccgtcgttgacctgcccgtcggcttgaacctgcaggaccagaccaccgctaccgtccgctcccgcatcacctctgctggtgcaggacagggacaggccgcttggttcgccaccttcaacgagacctttggtgactattccgaaaaggcacacgagctgctcaacaccaagctggagcagtgggccgaagaggccgtcgcccgtggcggattccacaacaccaccgccttgctcatccagtacgagaactaccgcgactggattgtcaaccacaacgtcgcgtactcggaactcttcctcgacactgccgacgtagccagcttcgatgtgtgggaccttctgcccttcacccgaggatacgttcacatcctcgacaaggacccctaccttcaccacttcgcctacgaccctcagtacttcctcaacgagctggacctgctcggtcaggctgccgctactcaactggcccgcaacatctccaactccggtgccatgcagacctacttcgctggggagactatccccggtgataacctcgcgtatgatgccgatttgagcgcctggactgagtacatcccgtaccacttccgtcctaactaccatggcgtgggtacttgctccatgatgccgaaggagatgggcggtgttgttgataatgctgcccgtgtgtatggtgtgcagggactgcgtgtcattgatggttctattcctcctacgcaaatgtcgtcccatgtcatgacggtgttctatgccatggcgctaaaaatttcggatgctatcttggaagattatgcttccatgcagtga

SEQ ID NO: 6 - DNA, 21 bp, synthetic construct
  source 1..21: mol_type = other DNA
atgcagactctccttgtgagc

SEQ ID NO: 7 - DNA, 23 bp, synthetic construct
  source 1..23: mol_type = other DNA
tcactgcatggaagcataatctt

SEQ ID NO: 8 - DNA, 26 bp, synthetic construct
  source 1..26: mol_type = other DNA
tatccatacgatgttcctgattatgc

SEQ ID NO: 9 - DNA, 33 bp, synthetic construct
  source 1..33: mol_type = other DNA
atactgtttaaattaatctatgctagcttattt

SEQ ID NO: 10 - DNA, 32 bp, synthetic construct
  source 1..32: mol_type = other DNA
gtgaataaaggcacctggactcgcccccacaa

SEQ ID NO: 11 - DNA, 36 bp, synthetic construct
  source 1..36: mol_type = other DNA
caggtgcctttattcactagagtagagccaccgaga

SEQ ID NO: 12 - DNA, 33 bp, synthetic construct
  source 1..33: mol_type = other DNA
aggaccccaaacttcaccacttcgcctacgacc

SEQ ID NO: 13 - DNA, 32 bp, synthetic construct
  source 1..32: mol_type = other DNA
gtgaagtttggggtccttgtcgaggatgtgaa

SEQ ID NO: 14 - DNA, 32 bp, synthetic construct
  source 1..32: mol_type = other DNA
gtgaatgacggcacctggactcgcccccacaa

SEQ ID NO: 15 - DNA, 36 bp, synthetic construct
  source 1..36: mol_type = other DNA
caggtgccgtcattcactagagtagagccaccgaga

SEQ ID NO: 16 - DNA, 33 bp, synthetic construct
  source 1..33: mol_type = other DNA
aggaccccgaccttcaccacttcgcctacgacc

SEQ ID NO: 17 - DNA, 32 bp, synthetic construct
  source 1..32: mol_type = other DNA
gtgaaggtcggggtccttgtcgaggatgtgaa